European Patent Application EP 4 292 661 A1, published December 20, 2023. Title: ANTI-VEGF ANTIBODY AND USE THEREOF. Applicant: SHANGHAIJEMINCARE PHARMACEUTICAL CO.,LTD；JIANGXI JEMINCARE GROUPCO.,LTD. The sequence listing filed with the application follows.

SEQUENCE LISTING (29 sequences)

SEQ ID NO: 1 - protein, 123 aa, Artificial Sequence
  Ab1910VE6 VH
AVQLVESGGGLVQAGGSARLSCAASGSTSDIVSMAWYRQAPGKERDLVAAVFAEDWRYVEDSVRGRFTISRDNTKNTVDLQMNNLKPEDTAIYYCNVRLRITDERRRERLDYWGQGTQVTVSS

SEQ ID NO: 2 - protein, 123 aa, Artificial Sequence
  Ab1910VE8 VH
EVQLVESGGGLVQPGGSLRLSCAASGSTSDIVSMAWYRQAPGKERELVSAVFAEDWRYVEDSVKGRFTISRDNSKNTVYLQMNSLRAEDTAVYYCNVRLRITDERRRERLDYWGKGTTVTVSS

SEQ ID NO: 3 - protein, 123 aa, Artificial Sequence
  Ab1910VE9 Ab1910VE18 VH
EVQLVESGGGLVQPGGSLRLSCAASGSTSDIVSMAWYRQAPGKERELVSAVFAEDWRYVEDSVKGRFTISRDNSKNTVYLQMNSLRAEDTAVYYCNVRLRITDERRRERLDYWGQGTLVTVSS

SEQ ID NO: 4 - protein, 123 aa, Artificial Sequence
  Ab1910VE21 VH
EVQLVESGGGLVQPGGSLRLSCAASGSTSDIVSMAWYRQAPGKERELVSAVLAPGWSYVEDSVKGRFTISRDNSKNTVYLQMNSLRAEDTAVYYCNVRLRITDERRRERLDYWGQGTLVTVSS

SEQ ID NO: 5 - protein, 123 aa, Artificial Sequence
  Ab1910VE23 VH
EVQLVESGGGLVQPGGSLRLSCAASGSTSDIVSMAWYRQAPGKERELVSAVFAEDWRYVEDSVKGRFTISRDNSKNTVYLQMNSLRAEDTAVYYCNVRLRIPHQWRTERLDYWGQGTLVTVSS

SEQ ID NO: 6 - protein, 123 aa, Artificial Sequence
  Ab1910VE24 VH
EVQLVESGGGLVQPGGSLRLSCAASGSTSDIVSMAWYRQAPGKERELVSAVFAEDWRYVEDSVKGRFTISRDNSKNTVYLQMNSLRAEDTAVYYCNVRLRITDWYSRERLDYWGQGTLVTVSS

SEQ ID NO: 7 - protein, 30 aa, Artificial Sequence
  Ab1910VE6 H-FR1
AVQLVESGGGLVQAGGSARLSCAASGSTSD

SEQ ID NO: 8 - protein, 30 aa, Artificial Sequence
  Ab1910VE8 Ab1910VE9 Ab1910VE18 Ab1910VE21 Ab1910VE23 Ab1910VE24 H-FR1
EVQLVESGGGLVQPGGSLRLSCAASGSTSD

SEQ ID NO: 9 - protein, 5 aa, Artificial Sequence
  HCDR1 HCDR1
IVSMA

SEQ ID NO: 10 - protein, 14 aa, Artificial Sequence
  Ab1910VE6  H-FR2
WYRQAPGKERDLVA

SEQ ID NO: 11 - protein, 14 aa, Artificial Sequence
  Ab1910VE8 Ab1910VE9 Ab1910VE18 Ab1910VE21 Ab1910VE23 Ab1910VE24 H-FR2
WYRQAPGKERELVS

SEQ ID NO: 12 - protein, 16 aa, Artificial Sequence
  Ab1910VE6  HCDR2
AVFAEDWRYVEDSVRG

SEQ ID NO: 13 - protein, 16 aa, Artificial Sequence
  Ab1910VE8 Ab1910VE9 Ab1910VE18 Ab1910VE23 Ab1910VE24  HCDR2
AVFAEDWRYVEDSVKG

SEQ ID NO: 14 - protein, 16 aa, Artificial Sequence
  Ab1910VE21  HCDR2
AVLAPGWSYVEDSVKG

SEQ ID NO: 15 - protein, 32 aa, Artificial Sequence
  Ab1910VE6  H-FR3
RFTISRDNTKNTVDLQMNNLKPEDTAIYYCNV

SEQ ID NO: 16 - protein, 32 aa, Artificial Sequence
  Ab1910VE8 Ab1910VE9 Ab1910VE18 Ab1910VE21 Ab1910VE23 Ab1910VE24 H-FR3
RFTISRDNSKNTVYLQMNSLRAEDTAVYYCNV

SEQ ID NO: 17 - protein, 15 aa, Artificial Sequence
  Ab1910VE6  Ab1910VE8 Ab1910VE9 Ab1910VE18 Ab1910VE21 HCDR3
RLRITDERRRERLDY

SEQ ID NO: 18 - protein, 15 aa, Artificial Sequence
  Ab1910VE23  HCDR3
RLRIPHQWRTERLDY

SEQ ID NO: 19 - protein, 15 aa, Artificial Sequence
  Ab1910VE24  HCDR3
RLRITDWYSRERLDY

SEQ ID NO: 20 - protein, 11 aa, Artificial Sequence
  Ab1910VE6  H-FR4
WGQGTQVTVSS

SEQ ID NO: 21 - protein, 11 aa, Artificial Sequence
  Ab1910VE8  H-FR4
WGKGTTVTVSS

SEQ ID NO: 22 - protein, 11 aa, Artificial Sequence
  Ab1910VE9 Ab1910VE18 Ab1910VE21 Ab1910VE23 Ab1910VE24  H-FR4
WGQGTLVTVSS

SEQ ID NO: 23 - protein, 16 aa, Artificial Sequence
  Ab1910VE6  HCDR2; Ab1910VE8 Ab1910VE9 Ab1910VE18 Ab1910VE23 Ab1910VE24  HCDR2; Ab1910VE21  HCDR2
  misc_feature (3)..(3): Xaa=Phe or Leu
  misc_feature (5)..(5): Xaa=Glu or Pro
  misc_feature (6)..(6): Xaa=Asp or Gly
  misc_feature (8)..(8): Xaa=Arg or Ser
  misc_feature (15)..(15): Xaa=Lys or Arg
AVXAXXWXYVEDSVXG

SEQ ID NO: 24 - protein, 15 aa, Artificial Sequence
  Ab1910VE6  Ab1910VE8 Ab1910VE9 Ab1910VE18 Ab1910VE21 HCDR3; Ab1910VE23  HCDR3; Ab1910VE24  HCDR3
  misc_feature (5)..(5): Xaa=Pro or Thr
  misc_feature (6)..(6): Xaa=Asp or His
  misc_feature (7)..(7): Xaa=Glu, Gln or Trp
  misc_feature (8)..(8): Xaa=Arg, Trp or Tyr
  misc_feature (9)..(9): Xaa=Arg or Ser
  misc_feature (10)..(10): Xaa=Arg or Thr
RLRIXXXXXXERLDY

SEQ ID NO: 25 - protein, 30 aa, Artificial Sequence
  Ab1910VE6 H-FR1; Ab1910VE8 Ab1910VE9 Ab1910VE18 Ab1910VE21 Ab1910VE23 Ab1910VE24 H-FR1
  misc_feature (1)..(1): Xaa=Ala or Glu
  misc_feature (14)..(14): Xaa=Ala or Pro
  misc_feature (18)..(18): Xaa=Ala or Leu
XVQLVESGGGLVQXGGSXRLSCAASGSTSD

SEQ ID NO: 26 - protein, 14 aa, Artificial Sequence
  Ab1910VE6  H-FR2; Ab1910VE8 Ab1910VE9 Ab1910VE18 Ab1910VE21 Ab1910VE23 Ab1910VE24 H-FR2
  misc_feature (11)..(11): Xaa=Asp or Glu
  misc_feature (14)..(14): Xaa=Ala or Ser
WYRQAPGKERXLVX

SEQ ID NO: 27 - protein, 32 aa, Artificial Sequence
  Ab1910VE6  H-FR3; Ab1910VE8 Ab1910VE9 Ab1910VE18 Ab1910VE21 Ab1910VE23 Ab1910VE24 H-FR3
  misc_feature (9)..(9): Xaa=Ser or Thr
  misc_feature (14)..(14): Xaa=Asp or Tyr
  misc_feature (19)..(19): Xaa=Asn or Ser
  misc_feature (21)..(21): Xaa=Lys or Arg
  misc_feature (22)..(22): Xaa=Ala or Pro
  misc_feature (27)..(27): Xaa=Ile or Val
RFTISRDNXKNTVXLQMNXLXXEDTAXYYCNV

SEQ ID NO: 28 - protein, 11 aa, Artificial Sequence
  Ab1910VE6  H-FR4; Ab1910VE8  H-FR4; Ab1910VE9 Ab1910VE18 Ab1910VE21 Ab1910VE23 Ab1910VE24  H-FR4
  misc_feature (3)..(3): Xaa=Lys or Gln
  misc_feature (6)..(6): Xaa=Leu, Gln or Thr
WGXGTXVTVSS

SEQ ID NO: 29 - protein, 123 aa, Artificial Sequence
  Ab1910VE6 VH; Ab1910VE8 VH; Ab1910VE9 Ab1910VE18 VH; Ab1910VE21 VH; Ab1910VE23 VH; Ab1910VE24 VH
  misc_feature (1)..(1): Xaa=Ala or Glu
  misc_feature (14)..(14): Xaa=Ala or Pro
  misc_feature (18)..(18): Xaa=Ala or Leu
  misc_feature (46)..(46): Xaa=Asp or Glu
  misc_feature (49)..(49): Xaa=Ala or Ser
  misc_feature (52)..(52): Xaa=Phe or Leu
  misc_feature (54)..(54): Xaa=Glu or Pro
  misc_feature (55)..(55): Xaa=Asp or Gly
  misc_feature (57)..(57): Xaa=Arg or Ser
  misc_feature (64)..(64): Xaa=Lys or Arg
  misc_feature (74)..(74): Xaa=Ser or Thr
  misc_feature (79)..(79): Xaa=Asp or Tyr
  misc_feature (84)..(84): Xaa=Asn or Ser
  misc_feature (86)..(86): Xaa=Lys or Arg
  misc_feature (87)..(87): Xaa=Ala or Pro
  misc_feature (92)..(92): Xaa=Ile or Val
  misc_feature (102)..(102): Xaa=Pro or Thr
  misc_feature (103)..(103): Xaa=Asp or His
  misc_feature (104)..(104): Xaa=Glu, Gln or Trp
  misc_feature (105)..(105): Xaa=Arg, Trp or Tyr
  misc_feature (106)..(106): Xaa=Arg or Ser
  misc_feature (107)..(107): Xaa=Arg or Thr
  misc_feature (115)..(115): Xaa=Lys or Gln
  misc_feature (118)..(118): Xaa=Leu, Gln or Thr
XVQLVESGGGLVQXGGSXRLSCAASGSTSDIVSMAWYRQAPGKERXLVXAVXAXXWXYVEDSVXGRFTISRDNXKNTVXLQMNXLXXEDTAXYYCNVRLRIXXXXXXERLDYWGXGTXVTVSS